European Patent Application EP 4 345 107 A2, published April 3, 2024. Title: RECOMBINANT FUSION PROTEINS AND LIBRARIES FROM IMMUNE CELL REPERTOIRES. Applicant: GIGAGEN, INC. The sequence listing filed with the application follows.

SEQUENCE LISTING (13 sequences)

SEQ ID NO: 1 - DNA, 4634 bp, synthetic construct
  misc_feature 1..4634: note = Description of Artificial Sequence: Synthetic polynucleotide
  source 1..4634: mol_type = other DNA
cttcagtaatgtcttgtttcttttgttgcagtggtgagccattttgacttcgtgaaagtttctttagaatagttgtttccagaggccaaacattccacccgtagtaaagtgcaagcgtaggaagaccaagactggcataaatcaggtataagtgtcgagcactggcaggtgatcttctgaaagtttctactagcagataagatccagtagtcatgcatatggcaacaatgtaccgtgtggatctaagaacgcgtcctactaaccttcgcattcgttggtccagtttgttgttatcgatcaacgtgacaaggttgtcgattccgcgtaagcatgcatacccaaggacgcctgttgcaattccaagtgagccagttccaacaatctttgtaatattagagcacttcattgtgttgcgcttgaaagtaaaatgcgaacaaattaagagataatctcgaaaccgcgacttcaaacgccaatatgatgtgcggcacacaataagcgttcatatccgctgggtgactttctcgctttaaaaaattatccgaaaaaattttctagagtgttgttactttatacttccggctcgtataatacgacaaggtgtaaggaggactaaaccatggctaaactcacctctgctgttccagtcctgactgctcgtgatgttgctggtgctgttgagttctggactgatagactcggtttctcccgtgacttcgtagaggacgactttgccggtgttgtacgtgacgacgttaccctgttcatctccgcagttcaggaccaggttgtgccagacaacactctggcatgggtatgggttcgtggtctggacgaactgtacgctgagtggtctgaggtcgtgtctaccaacttccgtgatgcatctggtccagctatgaccgagatcggtgaacagccctggggtcgtgagtttgcactgcgtgatccagctggtaactgcgtgcatttcgtcgcagaagaacaggactaacaattgacaccttacgattatttagagagtatttattagttttattgtatgtatacggatgttttattatctatttatgcccttatattctgtaactatccaaaagtcctatcttatcaagccagcaatctatgtccgcgaacgtcaactaaaaataagctttttatgctgttctctctttttttcccttcggtataattataccttgcatccacagattctcctgccaaattttgcataatcctttacaacatggctatatgggagcacttagcgccctccaaaacccatattgcctacgcatgtataggtgttttttccacaatattttctctgtgctctctttttattaaagagaagctctatatcggagaagcttctgtggccgttatattcggccttatcgtgggaccacattgcctgaattggtttgccccggaagattggggaaacttggatctgattaccttagctgcaggtaccactgagcgtcagaccccgtagaaaagatcaaaggatcttcttgagatcctttttttctgcgcgtaatctgctgcttgcaaacaaaaaaaccaccgctaccagcggtggtttgtttgccggatcaagagctaccaactctttttccgaaggtaactggcttcagcagagcgcagataccaaatactgttcttctagtgtagccgtagttaggccaccacttcaagaactctgtagcaccgcctacatacctcgctctgctaatcctgttaccagtggctgctgccagtggcgataagtcgtgtcttaccgggttggactcaagacgatagttaccggataaggcgcagcggtcgggctgaacggggggttcgtgcacacagcccagcttggagcgaacgacctacaccgaactgagatacctacagcgtgagctatgagaaagcgccacgcttcccgaagggagaaaggcggacaggtatccggtaagcggcagggtcggaacaggagagcgcacgagggagcttccagggggaaacgcctggtatctttatagtcctgtcgggtttcgccacctctgacttgagcgtcgatttttgtgatgctcgtcaggggggcggagcctatggaaaaacgccagcaacgcggcctttttacggttcctggccttttgctggccttttgctcacatgttctttcctgcggtacccagatccaattcccgctttgactgcctgaaatctccatcgcctacaatgatgacatttggatttggttgactcatgttggtattgtgaaatagacgcagatcgggaacactgaaaaatacacagttattattcatttaaataacatccaaagacgaaaggttgaatgaaacctttttgccatccgacatccacaggtccattctcacacataagtgccaaacgcaacaggaggggatacactagcagcagaccgttgcaaacgcaggacctccactcctcttctcctcaacacccacttttgccatcgaaaaaccagcccagttattgggcttgattggagctcgctcattccaattccttctattaggctactaacaccatgactttattagcctgtctatcctggcccccctggcgaggttcatgtttgtttatttccgaatgcaacaagctccgcattacacccgaacatcactccagatgagggctttctgagtgtggggtcaaatagtttcatgttccccaaatggcccaaaactgacagtttaaacgctgtcttggaacctaatatgacaaaagcgtgatctcatccaagatgaactaagtttggttcgttgaaatgctaacggccagttggtcaaaaagaaacttccaaaagtcggcataccgtttgtcttgtttggtattgattgacgaatgctcaaaaataatctcattaatgcttagcgcagtctctctatcgcttctgaaccccggtgcacctgtgccgaaacgcaaatggggaaacacccgctttttggatgattatgcattgtctccacattgtatgcttccaagattctggtgggaatactgctgatagcctaacgttcatgatcaaaatttaactgttctaacccctacttgacagcaatatataaacagaaggaagctgccctgtcttaaacctttttttttatcatcattattagcttactttcataattgcgactggttccaattgacaagcttttgattttaacgacttttaacgacaacttgagaagatcaaaaaacaactaattattgaaagaattccgaaacgatgagattcccatctattttcaccgctgtcttgttcgctgcctcctctgcattggctgcccctgttaacactaccactgaagacgagactgctcaaattccagctgaagcagttatcggttactctgaccttgagggtgatttcgacgtcgctgttttgcctttctctaactccactaacaacggtttgttgttcattaacaccactatcgcttccattgctgctaaggaagagggtgtctctctcgagaaaagagaggccgaagctgacatccagatgacccagtctccatcctccctgtctgcatctgtaggggacagagtcaccatcacttgtcgggcaagtcagggcatcagaaattacttagcctggtatcagcaaaaaccagggaaagcccctaagctcctgatctatgctgcatccactttgcaatcaggggtcccatctcggttcagtggcagtggatctgggacagatttcactctcaccatcagcagcctacagcctgaagatgttgcaacttattactgtcaaaggtataaccgtgcaccgtatacttttggccaggggaccaaggtggaaatcaaacgaactgtggctgcaccatctgtcggcggatcctctaggtcaagttccagcggcggcggtggcagcggaggcggcggtgaggtgcagctggtggagtctgggggaggcttggtacagcccggcaggtccctgagactctcctgtgcggcctctggattcacctttgatgattatgccatgcactgggtccggcaagctccagggaagggcctggaatgggtctcagctatcacttggaatagtggtcacatagactatgcggactctgtggagggccgattcaccatctccagagacaacgccaagaactccctgtatctgcaaatgaacagtctgagagctgaggatacggccgtatattactgtgcgaaagtctcgtaccttagcaccgcgtcctcccttgactattggggccaaggtaccctggtcaccgtctcgagtgcctccaccaagggcccatcggtcttcgaacagaagctcatctcagaagaggatctgtaaaggggcggccgctcaagaggatgtcagaatgccatttgcctgagagatgcaggcttcatttttgatacttttttatttgtaacctatatagtataggattttttttgtcattttgtttcttctcgtacgagcttgctcctgatcagcctatctcgcagcagatgaatatcttgtggtaggggtttgggaaaatcattcgagtttgatgtttttcttggtatttcccactcctcttcagagtacagaagattaagtgaaaccttcgtttgtgcggatc

SEQ ID NO: 2 - DNA, 7457 bp, synthetic construct
  misc_feature 1..7457: note = Description of Artificial Sequence: Synthetic polynucleotide
  source 1..7457: mol_type = other DNA
cttcagtaatgtcttgtttcttttgttgcagtggtgagccattttgacttcgtgaaagtttctttagaatagttgtttccagaggccaaacattccacccgtagtaaagtgcaagcgtaggaagaccaagactggcataaatcaggtataagtgtcgagcactggcaggtgatcttctgaaagtttctactagcagataagatccagtagtcatgcatatggcaacaatgtaccgtgtggatctaagaacgcgtcctactaaccttcgcattcgttggtccagtttgttgttatcgatcaacgtgacaaggttgtcgattccgcgtaagcatgcatacccaaggacgcctgttgcaattccaagtgagccagttccaacaatctttgtaatattagagcacttcattgtgttgcgcttgaaagtaaaatgcgaacaaattaagagataatctcgaaaccgcgacttcaaacgccaatatgatgtgcggcacacaataagcgttcatatccgctgggtgactttctcgctttaaaaaattatccgaaaaaattttctagagtgttgttactttatacttccggctcgtataatacgacaaggtgtaaggaggactaaaccatggctaaactcacctctgctgttccagtcctgactgctcgtgatgttgctggtgctgttgagttctggactgatagactcggtttctcccgtgacttcgtagaggacgactttgccggtgttgtacgtgacgacgttaccctgttcatctccgcagttcaggaccaggttgtgccagacaacactctggcatgggtatgggttcgtggtctggacgaactgtacgctgagtggtctgaggtcgtgtctaccaacttccgtgatgcatctggtccagctatgaccgagatcggtgaacagccctggggtcgtgagtttgcactgcgtgatccagctggtaactgcgtgcatttcgtcgcagaagaacaggactaacaattgacaccttacgattatttagagagtatttattagttttattgtatgtatacggatgttttattatctatttatgcccttatattctgtaactatccaaaagtcctatcttatcaagccagcaatctatgtccgcgaacgtcaactaaaaataagctttttatgctgttctctctttttttcccttcggtataattataccttgcatccacagattctcctgccaaattttgcataatcctttacaacatggctatatgggagcacttagcgccctccaaaacccatattgcctacgcatgtataggtgttttttccacaatattttctctgtgctctctttttattaaagagaagctctatatcggagaagcttctgtggccgttatattcggccttatcgtgggaccacattgcctgaattggtttgccccggaagattggggaaacttggatctgattaccttagctgcaggtaccactgagcgtcagaccccgtagaaaagatcaaaggatcttcttgagatcctttttttctgcgcgtaatctgctgcttgcaaacaaaaaaaccaccgctaccagcggtggtttgtttgccggatcaagagctaccaactctttttccgaaggtaactggcttcagcagagcgcagataccaaatactgttcttctagtgtagccgtagttaggccaccacttcaagaactctgtagcaccgcctacatacctcgctctgctaatcctgttaccagtggctgctgccagtggcgataagtcgtgtcttaccgggttggactcaagacgatagttaccggataaggcgcagcggtcgggctgaacggggggttcgtgcacacagcccagcttggagcgaacgacctacaccgaactgagatacctacagcgtgagctatgagaaagcgccacgcttcccgaagggagaaaggcggacaggtatccggtaagcggcagggtcggaacaggagagcgcacgagggagcttccagggggaaacgcctggtatctttatagtcctgtcgggtttcgccacctctgacttgagcgtcgatttttgtgatgctcgtcaggggggcggagcctatggaaaaacgccagcaacgcggcctttttacggttcctggccttttgctggccttttgctcacatgttctttcctgcggtacccagatccaattcccgctttgactgcctgaaatctccatcgcctacaatgatgacatttggatttggttgactcatgttggtattgtgaaatagacgcagatcgggaacactgaaaaatacacagttattattcatttaaataacatccaaagacgaaaggttgaatgaaacctttttgccatccgacatccacaggtccattctcacacataagtgccaaacgcaacaggaggggatacactagcagcagaccgttgcaaacgcaggacctccactcctcttctcctcaacacccacttttgccatcgaaaaaccagcccagttattgggcttgattggagctcgctcattccaattccttctattaggctactaacaccatgactttattagcctgtctatcctggcccccctggcgaggttcatgtttgtttatttccgaatgcaacaagctccgcattacacccgaacatcactccagatgagggctttctgagtgtggggtcaaatagtttcatgttccccaaatggcccaaaactgacagtttaaacgctgtcttggaacctaatatgacaaaagcgtgatctcatccaagatgaactaagtttggttcgttgaaatgctaacggccagttggtcaaaaagaaacttccaaaagtcggcataccgtttgtcttgtttggtattgattgacgaatgctcaaaaataatctcattaatgcttagcgcagtctctctatcgcttctgaaccccggtgcacctgtgccgaaacgcaaatggggaaacacccgctttttggatgattatgcattgtctccacattgtatgcttccaagattctggtgggaatactgctgatagcctaacgttcatgatcaaaatttaactgttctaacccctacttgacagcaatatataaacagaaggaagctgccctgtcttaaacctttttttttatcatcattattagcttactttcataattgcgactggttccaattgacaagcttttgattttaacgacttttaacgacaacttgagaagatcaaaaaacaactaattattgaaagaattccgaaacgatgagattcccatctattttcaccgctgtcttgttcgctgcctcctctgcattggctgcccctgttaacactaccactgaagacgagactgctcaaattccagctgaagcagttatcggttactctgaccttgagggtgatttcgacgtcgctgttttgcctttctctaactccactaacaacggtttgttgttcattaacaccactatcgcttccattgctgctaaggaagagggtgtctctctcgagaaaagagaggccgaagctgacatccagatgacccagtctccatcctccctgtctgcatctgtaggggacagagtcaccatcacttgtcgggcaagtcagggcatcagaaattacttagcctggtatcagcaaaaaccagggaaagcccctaagctcctgatctatgctgcatccactttgcaatcaggggtcccatctcggttcagtggcagtggatctgggacagatttcactctcaccatcagcagcctacagcctgaagatgttgcaacttattactgtcaaaggtataaccgtgcaccgtatacttttggccaggggaccaaggtggaaatcaaacgaactgtggctgcaccatctgtcttcatcttcccgccatctgatgagcagttgaaatctggaactgcctctgttgtgtgcctgctgaataacttctatcccagagaggccaaagtacagtggaaggtggataacgccctccaatcgggtaactcccaggagagtgtcacagagcaggacagcaaggacagcacctacagcctcagcagcaccctgacgctgagcaaagcagactacgagaaacacaaagtctacgcctgcgaagtcacccatcagggcctgagctcgcccgtcacaaagagcttcaacaggggagagtgttaaaggggcggccgctcaagaggatgtcagaatgccatttgcctgagagatgcaggcttcatttttgatacttttttatttgtaacctatatagtataggattttttttgtcattttgtttcttctcgtacgagcttgctcctgatcagcctatctcgcagcagatgaatatcttgtggtaggggtttgggaaaatcattcgagtttgatgtttttcttggtatttcccactcctcttcagagtacagaagattaagtgaaaccttcgtttgtgcgtgttctttcctgcggtacccagatccaattcccgctttgactgcctgaaatctccatcgcctacaatgatgacatttggatttggttgactcatgttggtattgtgaaatagacgcagatcgggaacactgaaaaatacacagttattattcatttaaataacatccaaagacgaaaggttgaatgaaacctttttgccatccgacatccacaggtccattctcacacataagtgccaaacgcaacaggaggggatacactagcagcagaccgttgcaaacgcaggacctccactcctcttctcctcaacacccacttttgccatcgaaaaaccagcccagttattgggcttgattggagctcgctcattccaattccttctattaggctactaacaccatgactttattagcctgtctatcctggcccccctggcgaggttcatgtttgtttatttccgaatgcaacaagctccgcattacacccgaacatcactccagatgagggctttctgagtgtggggtcaaatagtttcatgttccccaaatggcccaaaactgacagtttaaacgctgtcttggaacctaatatgacaaaagcgtgatctcatccaagatgaactaagtttggttcgttgaaatgctaacggccagttggtcaaaaagaaacttccaaaagtcggcataccgtttgtcttgtttggtattgattgacgaatgctcaaaaataatctcattaatgcttagcgcagtctctctatcgcttctgaaccccggtgcacctgtgccgaaacgcaaatggggaaacacccgctttttggatgattatgcattgtctccacattgtatgcttccaagattctggtgggaatactgctgatagcctaacgttcatgatcaaaatttaactgttctaacccctacttgacagcaatatataaacagaaggaagctgccctgtcttaaacctttttttttatcatcattattagcttactttcataattgcgactggttccaattgacaagcttttgattttaacgacttttaacgacaacttgagaagatcaaaaaacaactaattattgaaagaattccgaaacgatgagattcccatctattttcaccgctgtcttgttcgctgcctcctctgcattggctgcccctgttaacactaccactgaagacgagactgctcaaattccagctgaagcagttatcggttactctgaccttgagggtgatttcgacgtcgctgttttgcctttctctaactccactaacaacggtttgttgttcattaacaccactatcgcttccattgctgctaaggaagagggtgtctctctcgagaaaagagaggccgaagctgaggtgcagctggtggagtctgggggaggcttggtacagcccggcaggtccctgagactctcctgtgcggcctctggattcacctttgatgattatgccatgcactgggtccggcaagctccagggaagggcctggaatgggtctcagctatcacttggaatagtggtcacatagactatgcggactctgtggagggccgattcaccatctccagagacaacgccaagaactccctgtatctgcaaatgaacagtctgagagctgaggatacggccgtatattactgtgcgaaagtctcgtaccttagcaccgcgtcctcccttgactattggggccaaggtaccctggtcaccgtctcgagtgcctccaccaagggcccatcggtcttccccctggcaccctcctccaagagcacctctgggggcacagcggccctgggctgcctggtcaaggactacttccccgaaccggtgacggtgtcgtggaactcaggcgccctgaccagcggcgtgcacaccttcccggctgtcctacagtcctcaggactctactccctcagcagcgtggtgaccgtgccctccagcagcttgggcacccagacctacatctgcaacgtgaatcacaagcccagcaacaccaaggtggacaagaaagttgagcccaaatcttgtgacaaaactcacacatgcccaccgtgcccagcacctgaactcctggggggaccgtcagtcttcctcttccccccaaaacccaaggacaccctcatgatctcccggacccctgaggtcacatgcgtggtggtggacgtgagccacgaagaccctgaggtcaagttcaactggtacgtggacggcgtggaggtgcataatgccaagacaaagccgcgggaggagcagtacaacagcacgtaccgtgtggtcagcgtcctcaccgtcctgcaccaggactggctgaatggcaaggagtacaagtgcaaggtctccaacaaagccctcccagcccccatcgagaaaaccatctccaaagccaaagggcagccccgagaaccacaggtgtacaccctgcccccatcccgggatgagctgaccaagaaccaggtcagcctgacctgcctggtcaaaggcttctatcccagcgacatcgccgtggagtgggagagcaatgggcagccggagaacaactacaagaccacgcctcccgtgctggactccgacggctccttcttcctctacagcaagctcaccgtggacaagagcaggtggcagcaggggaacgtcttctcatgctccgtgatgcatgaggctctgcacaaccactacacgcagaagagcctctccctgtctccgggtaaataaaggggcggccgctcaagaggatgtcagaatgccatttgcctgagagatgcaggcttcatttttgatacttttttatttgtaacctatatagtataggattttttttgtcattttgtttcttctcgtacgagcttgctcctgatcagcctatctcgcagcagatgaatatcttgtggtaggggtttgggaaaatcattcgagtttgatgtttttcttggtatttcccactcctcttcagagtacagaagattaagtgaaaccttcgtttgtgcggatc

SEQ ID NO: 3 - DNA, 1944 bp, synthetic construct
  misc_feature 1..1944: note = Description of Artificial Sequence: Synthetic polynucleotide
  source 1..1944: mol_type = other DNA
ttcatcttcccgccatctgatgagcagttgaaatctggaactgcctctgttgtgtgcctgctgaataacttctatcccagagaggccaaagtacagtggaaggtggataacgccctccaatcgggtaactcccaggagagtgtcacagagcaggacagcaaggacagcacctacagcctcagcagcaccctgacgctgagcaaagcagactacgagaaacacaaagtctacgcctgcgaagtcacccatcagggcctgagctcgcccgtcacaaagagcttcaacaggggagagtgttaaaggggcggccgctcaagaggatgtcagaatgccatttgcctgagagatgcaggcttcatttttgatacttttttatttgtaacctatatagtataggattttttttgtcattttgtttcttctcgtacgagcttgctcctgatcagcctatctcgcagcagatgaatatcttgtggtaggggtttgggaaaatcattcgagtttgatgtttttcttggtatttcccactcctcttcagagtacagaagattaagtgaaaccttcgtttgtgcgtgttctttcctgcggtacccagatccaattcccgctttgactgcctgaaatctccatcgcctacaatgatgacatttggatttggttgactcatgttggtattgtgaaatagacgcagatcgggaacactgaaaaatacacagttattattcatttaaataacatccaaagacgaaaggttgaatgaaacctttttgccatccgacatccacaggtccattctcacacataagtgccaaacgcaacaggaggggatacactagcagcagaccgttgcaaacgcaggacctccactcctcttctcctcaacacccacttttgccatcgaaaaaccagcccagttattgggcttgattggagctcgctcattccaattccttctattaggctactaacaccatgactttattagcctgtctatcctggcccccctggcgaggttcatgtttgtttatttccgaatgcaacaagctccgcattacacccgaacatcactccagatgagggctttctgagtgtggggtcaaatagtttcatgttccccaaatggcccaaaactgacagtttaaacgctgtcttggaacctaatatgacaaaagcgtgatctcatccaagatgaactaagtttggttcgttgaaatgctaacggccagttggtcaaaaagaaacttccaaaagtcggcataccgtttgtcttgtttggtattgattgacgaatgctcaaaaataatctcattaatgcttagcgcagtctctctatcgcttctgaaccccggtgcacctgtgccgaaacgcaaatggggaaacacccgctttttggatgattatgcattgtctccacattgtatgcttccaagattctggtgggaatactgctgatagcctaacgttcatgatcaaaatttaactgttctaacccctacttgacagcaatatataaacagaaggaagctgccctgtcttaaacctttttttttatcatcattattagcttactttcataattgcgactggttccaattgacaagcttttgattttaacgacttttaacgacaacttgagaagatcaaaaaacaactaattattgaaagaattccgaaacgatgagattcccatctattttcaccgctgtcttgttcgctgcctcctctgcattggctgcccctgttaacactaccactgaagacgagactgctcaaattccagctgaagcagttatcggttactctgaccttgagggtgatttcgacgtcgctgttttgcctttctctaactccactaacaacggtttgttgttcattaacaccactatcgcttccattgctgctaaggaagagggtgtctctctcgagaaaagagaggccgaagct

SEQ ID NO: 4 - DNA, 48 bp, synthetic construct
  misc_feature 1..48: note = Description of Artificial Sequence: Synthetic primer
  source 1..48: mol_type = other DNA
gtctctctcgagaaaagagaggccgaagctsaggtgcagctggtggag

SEQ ID NO: 5 - DNA, 51 bp, synthetic construct
  misc_feature 1..51: note = Description of Artificial Sequence: Synthetic primer
  source 1..51: mol_type = other DNA
caactgctcatcagatggcgggaagatgaagacagatggtgcagccacagt

SEQ ID NO: 6 - DNA, 35 bp, synthetic construct
  misc_feature 1..35: note = Description of Artificial Sequence: Synthetic probe
  source 1..35: mol_type = other DNA
ctgccacctgctcttgtccacggtgagcttgctgt

SEQ ID NO: 7 - DNA, 35 bp, synthetic construct
  misc_feature 1..35: note = Description of Artificial Sequence: Synthetic probe
  source 1..35: mol_type = other DNA
tgatgggtgacttcgcaggcgtagagtttgtgttt

SEQ ID NO: 8 - DNA, 27 bp, synthetic construct
  misc_feature 1..27: note = Description of Artificial Sequence: Synthetic primer
  source 1..27: mol_type = other DNA
ggactggacatccagwtgacccagtct

SEQ ID NO: 9 - DNA, 54 bp, synthetic construct
  misc_feature 1..54: note = Description of Artificial Sequence: Synthetic primer
  source 1..54: mol_type = other DNA
gccgccgctggaacttgacctagaggatccgccgacagatggtgcagccacagt

SEQ ID NO: 10 - DNA, 60 bp, synthetic construct
  misc_feature 1..60: note = Description of Artificial Sequence: Synthetic primer
  source 1..60: mol_type = other DNA
aggtcaagttccagcggcggcggtggcagcggaggcggcggtsaggtgcagctggtggag

SEQ ID NO: 11 - DNA, 20 bp, synthetic construct
  misc_feature 1..20: note = Description of Artificial Sequence: Synthetic primer
  source 1..20: mol_type = other DNA
ccryggctttgtcttggcat

SEQ ID NO: 12 - DNA, 8956 bp, synthetic construct
  misc_feature 1..8956: note = Description of Artificial Sequence: Synthetic polynucleotide
  source 1..8956: mol_type = other DNA
agatctaacatccaaagacgaaaggttgaatgaaacctttttgccatccgacatccacaggtccattctcacacataagtgccaaacgcaacaggaggggatacactagcagcagaccgttgcaaacgcaggacctccactcctcttctcctcaacacccacttttgccatcgaaaaaccagcccagttattgggcttgattggagctcgctcattccaattccttctattaggctactaacaccatgactttattagcctgtctatcctggcccccctggcgaggttcatgtttgtttatttccgaatgcaacaagctccgcattacacccgaacatcactccagatgagggctttctgagtgtggggtcaaatagtttcatgttccccaaatggcccaaaactgacagtttaaacgctgtcttggaacctaatatgacaaaagcgtgatctcatccaagatgaactaagtttggttcgttgaaatgctaacggccagttggtcaaaaagaaacttccaaaagtcgccataccgtttgtcttgtttggtattgattgacgaatgctcaaaaataatctcattaatgcttagcgcagtctctctatcgcttctgaaccccggtgcacctgtgccgaaacgcaaatggggaaacacccgctttttggatgattatgcattgtctccacattgtatgcttccaagattctggtgggaatactgctgatagcctaacgttcatgatcaaaatttaactgttctaacccctacttgacagcaatatataaacagaaggaagctgccctgtcttaaacctttttttttatcatcattattagcttactttcataattgcgactggttccaattgacaagcttttgattttaacgacttttaacgacaacttgagaagatcaaaaaacaactaattattcgaaggatccaaacgatgagatttccttcaatttttactgcagttttattcgcagcatcctccgcattagctgctccagtcaacactacaacagaagatgaaacggcacaaattccggctgaagctgtcatcggttactcagatttagaaggggatttcgatgttgctgttttgccattttccaacagcacaaataacgggttattgtttataaatactactattgccagcattgctgctaaagaagaaggggtatctctcgagaaaagagaggctgaagctcccctggcaccctcctccaagagcacctctgggggcacagcggccctgggctgcctggtcaaggactacttccccgaaccggtgacggtgtcgtggaactcaggcgccctgaccagcggcgtgcacaccttcccggctgtcctacagtcctcaggactctactccctcagcagcgtggtgaccgtgccctccagcagcttgggcacccagacctacatctgcaacgtgaatcacaagcccagcaacaccaaggtggacaagaaagttgagcccaaatcttgtgacaaaactcacacatgcccaccgtgcccagcacctgaactcctggggggaccgtcagtcttcctcttccccccaaaacccaaggacaccctcatgatctcccggacccctgaggtcacatgcgtggtggtggacgtgagccacgaagaccctgaggtcaagttcaactggtacgtggacggcgtggaggtgcataatgccaagacaaagccgcgggaggagcagtacaacagcacgtaccgtgtggtcagcgtcctcaccgtcctgcaccaggactggctgaatggcaaggagtacaagtgcaaggtctccaacaaagccctcccagcccccatcgagaaaaccatctccaaagccaaagggcagccccgagaaccacaggtgtacaccctgcccccatcccgggatgagctgaccaagaaccaggtcagcctgacctgcctggtcaaaggcttctatcccagcgacatcgccgtggagtgggagagcaatgggcagccggagaacaactacaagaccacgcctcccgtgctggactccgacggctccttcttcctctacagcaagctcaccgtggacaagagcaggtggcagcaggggaacgtcttctcatgctccgtgatgcatgaggctctgcacaaccactacacgcagaagagcctctccctgtctccgggtaaataattcgccttagacatgactgttcctcagttcaagttgggcacttacgagaagaccggtcttgctagattctaatcaagaggatgtcagaatgccatttgcctgagagatgcaggcttcatttttgatacttttttatttgtaacctatatagtataggattttttttgtcattttgtttcttctcgtacgagcttgctcctgatcagcctatctcgcagctgatgaatatcttgtggtaggggtttgggaaaatcattcgagtttgatgtttttcttggtatttcccactcctcttcagagtacagaagattaagtgagaagttcgtttgtgcaagcttatcgataagctttaatgcggtagtttatcacagttaaattgctaacgcagtcaggcaccgtgtatgaaatctaacaatgcgctcatcgtcatcctcggcaccgtcaccctggatgctgtaggcataggcttggttatgccggtactgccgggcctcttgcgggatatcgtccattccgacagcatcgccagtcactatggcgtgctgctagcgctatatgcgttgatgcaatttctatgcgcacccgttctcggagcactgtccgaccgctttggccgccgcccagtcctgctcgcttcgctacttggagccactatcgactacgcgatcatggcgaccacacccgtcctgtggatctatcgaatctaaatgtaagttaaaatctctaaataattaaataagtcccagtttctccatacgaaccttaacagcattgcggtgagcatctagaccttcaacagcagccagatccatcactgcttggccaatatgtttcagtccctcaggagttacgtcttgtgaagtgatgaacttctggaaggttgcagtgttaactccgctgtattgacgggcatatccgtacgttggcaaagtgtggttggtaccggaggagtaatctccacaactctctggagagtaggcaccaacaaacacagatccagcgtgttgtacttgatcaacataagaagaagcattctcgatttgcaggatcaagtgttcaggagcgtactgattggacatttccaaagcctgctcgtaggttgcaaccgatagggttgtagagtgtgcaatacacttgcgtacaatttcaacccttggcaactgcacagcttggttgtgaacagcatcttcaattctggcaagctccttgtctgtcatatcgacagccaacagaatcacctgggaatcaataccatgttcagcttgagacagaaggtctgaggcaacgaaatctggatcagcgtatttatcagcaataactagaacttcagaaggcccagcaggcatgtcaatactacacagggctgatgtgtcattttgaaccatcatcttggcagcagtaacgaactggtttcctggaccaaatattttgtcacacttaggaacagtttctgttccgtaagccatagcagctactgcctgggcgcctcctgctagcacgatacacttagcaccaaccttgtgggcaacgtagatgacttctggggtaagggtaccatccttcttaggtggagatgcaaaaacaatttctttgcaaccagcaactttggcaggaacacccagcatcagggaagtggaaggcagaattgcggttccaccaggaatatagaggccaactttctcaataggtcttgcaaaacgagagcagactacaccagggcaagtctcaacttgcaacgtctccgttagttgagcttcatggaatttcctgacgttatctatagagagatcaatggctctcttaacgttatctggcaattgcataagttcctctgggaaaggagcttctaacacaggtgtcttcaaagcgactccatcaaacttggcagttagttctaaaagggctttgtcaccattttgacgaacattgtcgacaattggtttgactaattccataatctgttccgttttctggataggacgacgaagggcatcttcaatttcttgtgaggaggccttagaaacgtcaattttgcacaattcaatacgaccttcagaagggacttctttaggtttggattcttctttaggttgttccttggtgtatcctggcttggcatctcctttccttctagtgacctttagggacttcatatccaggtttctctccacctcgtccaacgtcacaccgtacttggcacatctaactaatgcaaaataaaataagtcagcacattcccaggctatatcttccttggatttagcttctgcaagttcatcagcttcctccctaattttagcgttcaacaaaacttcgtcgtcaaataaccgtttggtataagaaccttctggagcattgctcttacgatcccacaaggtggcttccatggctctaagaccctttgattggccaaaacaggaagtgcgttccaagtgacagaaaccaacacctgtttgttcaaccacaaatttcaagcagtctccatcacaatccaattcgatacccagcaacttttgagttgctccagatgtagcacctttataccacaaaccgtgacgacgagattggtagactccagtttgtgtccttatagcctccggaatagactttttggacgagtacaccaggcccaacgagtaattagaagagtcagccaccaaagtagtgaatagaccatcggggcggtcagtagtcaaagacgccaacaaaatttcactgacagggaactttttgacatcttcagaaagttcgtattcagtagtcaattgccgagcatcaataatggggattataccagaagcaacagtggaagtcacatctaccaactttgcggtctcagaaaaagcataaacagttctactaccgccattagtgaaacttttcaaatcgcccagtggagaagaaaaaggcacagcgatactagcattagcgggcaaggatgcaactttatcaaccagggtcctatagataaccctagcgcctgggatcatcctttggacaactctttctgccaaatctaggtccaaaatcacttcattgataccattattgtacaacttgagcaagttgtcgatcagctcctcaaattggtcctctgtaacggatgactcaacttgcacattaacttgaagctcagtcgattgagtgaacttgatcaggttgtgcagctggtcagcagcatagggaaacacggcttttcctaccaaactcaaggaattatcaaactctgcaacacttgcgtatgcaggtagcaagggaaatgtcatacttgaagtcggacagtgagtgtagtcttgagaaattctgaagccgtatttttattatcagtgagtcagtcatcaggagatcctctacgccggacgcatcgtggccggcatcaccggcgccacaggtgcggttgctggcgcctatatcgccgacatcaccgatggggaagatcgggctcgccacttcgggctcatgagcgcttgtttcggcgtgggtatggtggcaggccccgtggccgggggactgttgggcgccatctccttgcatgcaccattccttgcggcggcggtgctcaacggcctcaacctactactgggctgcttcctaatgcaggagtcgcataagggagagcgtcgagtatctatgattggaagtatgggaatggtgatacccgcattcttcagtgtcttgaggtctcctatcagattatgcccaactaaagcaaccggaggaggagatttcatggtaaatttctctgacttttggtcatcagtagactcgaactgtgagactatctcggttatgacagcagaaatgtccttcttggagacagtaaatgaagtcccaccaataaagaaatccttgttatcaggaacaaacttcttgtttcgaactttttcggtgccttgaactataaaatgtagagtggatatgtcgggtaggaatggagcgggcaaatgcttaccttctggaccttcaagaggtatgtagggtttgtagatactgatgccaacttcagtgacaacgttgctatttcgttcaaaccattccgaatccagagaaatcaaagttgtttgtctactattgatccaagccagtgcggtcttgaaactgacaatagtgtgctcgtgttttgaggtcatctttgtatgaataaatctagtctttgatctaaataatcttgacgagccaaggcgataaatacccaaatctaaaactcttttaaaacgttaaaaggacaagtatgtctgcctgtattaaaccccaaatcagctcgtagtctgatcctcatcaacttgaggggcactatcttgttttagagaaatttgcggagatgcgatatcgagaaaaaggtacgctgattttaaacgtgaaatttatctcaagatctctgcctcgcgcgtttcggtgatgacggtgaaaacctctgacacatgcagctcccggagacggtcacagcttgtctgtaagcggatgccgggagcagacaagcccgtcagggcgcgtcagcgggtgttggcgggtgtcggggcgcagccatgacccagtcacgtagcgatagcggagtgtatactggcttaactatgcggcatcagagcagattgtactgagagtgcaccatatgcggtgtgaaataccgcacagatgcgtaaggagaaaataccgcatcaggcgctcttccgcttcctcgctcactgactcgctgcgctcggtcgttcggctgcggcgagcggtatcagctcactcaaaggcggtaatacggttatccacagaatcaggggataacgcaggaaagaacatgtgagcaaaaggccagcaaaaggccaggaaccgtaaaaaggccgcgttgctggcgtttttccataggctccgcccccctgacgagcatcacaaaaatcgacgctcaagtcagaggtggcgaaacccgacaggactataaagataccaggcgtttccccctggaagctccctcgtgcgctctcctgttccgaccctgccgcttaccggatacctgtccgcctttctcccttcgggaagcgtggcgctttctcaatgctcacgctgtaggtatctcagttcggtgtaggtcgttcgctccaagctgggctgtgtgcacgaaccccccgttcagcccgaccgctgcgccttatccggtaactatcgtcttgagtccaacccggtaagacacgacttatcgccactggcagcagccactggtaacaggattagcagagcgaggtatgtaggcggtgctacagagttcttgaagtggtggcctaactacggctacactagaaggacagtatttggtatctgcgctctgctgaagccagttaccttcggaaaaagagttggtagctcttgatccggcaaacaaaccaccgctggtagcggtggtttttttgtttgcaagcagcagattacgcgcagaaaaaaaggatctcaagaagatcctttgatcttttctacggggtctgacgctcagtggaacgaaaactcacgttaagggattttggtcatgagattatcaaaaaggatcttcacctagatccttttaaattaaaaatgaagttttaaatcaatctaaagtatatatgagtaaacttggtctgacagttaccaatgcttaatcagtgaggcacctatctcagcgatctgtctatttcgttcatccatagttgcctgactccccgtcgtgtagataactacgatacgggagggcttaccatctggccccagtgctgcaatgataccgcgagacccacgctcaccggctccagatttatcagcaataaaccagccagccggaagggccgagcgcagaagtggtcctgcaactttatccgcctccatccagtctattaattgttgccgggaagctagagtaagtagttcgccagttaatagtttgcgcaacgttgttgccattgctgcaggcatcgtggtgtcacgctcgtcgtttggtatggcttcattcagctccggttcccaacgatcaaggcgagttacatgatcccccatgttgtgcaaaaaagcggttagctccttcggtcctccgatcgttgtcagaagtaagttggccgcagtgttatcactcatggttatggcagcactgcataattctcttactgtcatgccatccgtaagatgcttttctgtgactggtgagtactcaaccaagtcattctgagaatagtgtatgcggcgaccgagttgctcttgcccggcgtcaacacgggataataccgcgccacatagcagaactttaaaagtgctcatcattggaaaacgttcttcggggcgaaaactctcaaggatcttaccgctgttgagatccagttcgatgtaacccactcgtgcacccaactgatcttcagcatcttttactttcaccagcgtttctgggtgagcaaaaacaggaaggcaaaatgccgcaaaaaagggaataagggcgacacggaaatgttgaatactcatactcttcctttttcaatattattgaagcatttatcagggttattgtctcatgagcggatacatatttgaatgtatttagaaaaataaacaaataggggttccgcgcacatttccccgaaaagtgccacctgacgtctaagaaaccattattatcatgacattaacctataaaaataggcgtatcacgaggccctttcgtcttcaagaattaattctcatgtttgacagcttatcatcgataagctgactcatgttggtattgtgaaatagacgcagatcgggaacactgaaaaataacagttattattcg

SEQ ID NO: 13 - DNA, 789 bp, synthetic construct
  misc_feature 1..789: note = Description of Artificial Sequence: Synthetic polynucleotide
  source 1..789: mol_type = other DNA
gacatccagatgacccagtctccatcctccctgtctgcatctgtaggggacagagtcaccatcacttgtcgggcaagtcagggcatcagaaattacttagcctggtatcagcaaaaaccagggaaagcccctaagctcctgatctatgctgcatccactttgcaatcaggggtcccatctcggttcagtggcagtggatctgggacagatttcactctcaccatcagcagcctacagcctgaagatgttgcaacttattactgtcaaaggtataaccgtgcaccgtatacttttggccaggggaccaaggtggaaatcaaacgaactgtggctgcaccatctgtcggcggatcctctaggtcaagttccagcggcggcggtggcagcggaggcggcggtgaggtgcagctggtggagtctgggggaggcttggtacagcccggcaggtccctgagactctcctgtgcggcctctggattcacctttgatgattatgccatgcactgggtccggcaagctccagggaagggcctggaatgggtctcagctatcacttggaatagtggtcacatagactatgcggactctgtggagggccgattcaccatctccagagacaacgccaagaactccctgtatctgcaaatgaacagtctgagagctgaggatacggccgtatattactgtgcgaaagtctcgtaccttagcaccgcgtcctcccttgactattggggccaaggtaccctggtcaccgtctcgagtgcctccaccaagggcccatcggtcttc